European Patent Specification EP 3 403 658 B1, published August 9, 2023. Title: A Composition for Treating Ischemic Diseases or Neuroinflammatory Diseases Comprising Neural Precursor Cells or Therir Secretome. Applicant: S-BIOMEDICS. Application 15812792.8. The sequence listing filed with the application follows.

SEQUENCE LISTING (2 sequences)

SEQ ID NO: 1 - DNA, 22 bp, Artificial Sequence
  forward primer for Angiopoietin-1
tgtgtccatcagctccagttgc

SEQ ID NO: 2 - DNA, 22 bp, Artificial Sequence
  reverse primer for Angiopoietin-1
cggctaccatgctcgagatagg